European Patent Specification EP 3 265 198 B1, published April 26, 2023. Title: SANITIZATION METHOD FOR AFFINITY CHROMATOGRAPHY MATRICES. Applicant: GE Healthcare Bio-Sciences AB. The sequence listing filed with the application follows.

SEQUENCE LISTING (19 sequences)

SEQ ID NO: 1 - protein, 51 aa, Staphylococcus aureus
AQQNAFYQVLNMPNLNADQRNGFIQSLKDDPSQSANVLGEAQKLNDSQAPK

SEQ ID NO: 2 - protein, 61 aa, Staphylococcus aureus
ADAQQNKFNKDQQSAFYEILNMPNLNEEQRNGFIQSLKDDPSQSTNVLGEAKKLNESQAPK

SEQ ID NO: 3 - protein, 58 aa, Staphylococcus aureus
ADNNFNKEQQNAFYEILNMPNLNEEQRNGFIQSLKDDPSQSANLLAEAKKLNESQAPK

SEQ ID NO: 4 - protein, 58 aa, Staphylococcus aureus [sequence omitted]

SEQ ID NO: 5 - protein, 58 aa, Staphylococcus aureus
ADNKFNKEQQNAFYEILHLPNLTEEQRNGFIQSLKDDPSVSKEILAEAKKLNDAQAPK

SEQ ID NO: 6 - protein, 58 aa, Escherichia coli [sequence omitted]

SEQ ID NO: 7 - protein, 72 aa, Peptostreptococcus magnus
SEEEVTIKANLIFANGSTQTAEFKGTFEKATSEAYAYADTLKKDNGEYTVDVADKGYTLNIKFAGKEKTPEE

SEQ ID NO: 8 - protein, 72 aa, Peptostreptococcus magnus
PKEEVTIKANLIYADGKTQTAEFKGTFEEATAEAYRYADALKKDNGEYTVDVADKGYTLNIKFAGKEKTPEE

SEQ ID NO: 9 - protein, 72 aa, Peptostreptococcus magnus
PKEEVTIKANLIYADGKTQTAEFKGTFEEATAEAYRYADLLAKENGKYTVDVADKGYTLNIKFAGKEKTPEE

SEQ ID NO: 10 - protein, 74 aa, Peptostreptococcus magnus
PKEEVTIKANLIYADGKTQTAEFKGTFAEATAEAYRYADLLAKENGKYTADLEDGGYTINIRFAGKKVDEKPEE

SEQ ID NO: 11 - protein, 65 aa, Peptostreptococcus magnus
EKEQVTIKENIYFEDGTVQTATFKGTFAEATAEAYRYADLLSKEHGKYTADLEDGGYTINIRFAG

SEQ ID NO: 12 - protein, 58 aa, Escherichia coli
VDNKFNKEQQNAFYEILHLPNLTEEQRNAFIQSLKDDPSQSANLLAEAKKLNDAQAPK

SEQ ID NO: 13 - protein, 58 aa, Escherichia coli [sequence omitted]

SEQ ID NO: 14 - protein, 58 aa, Escherichia coli
ADNKFNKEQQNAFYEILHLPNLTEEQRNAFIQSLKDDPSVSKEILAEAKKLNDAQAPK

SEQ ID NO: 15 - protein, 58 aa, Escherichia coli
ADNKFNKEQQNAFYEILHLPNLTEEQRNAFIQELKDDPSVSKEILAEAKKLNDAQAPK

SEQ ID NO: 16 - protein, 54 aa, Escherichia coli
FNKEQQNAFYEILHLPNLTEEQRNGFIQSLKDDPSVSKEILAEAKKLNDAQAPK

SEQ ID NO: 17 - protein, 286 aa, Staphylococcus aureus
AQQNAFYQVLNMPNLNADQRNGFIQSLKDDPSQSANVLGEAQKLNDSQAPKADAQQNKFNKDQQSAFYEILNMPNLNEEQRNGFIQSLKDDPSQSTNVLGEAKKLNESQAPKADNNFNKEQQNAFYEILNMPNLNEEQRNGFIQSLKDDPSQSANLLAEAKKLNESQAPKADNKFNKEQQNAFYEILHLPNLNEEQRNGFIQSLKDDPSQSANLLAEAKKLNDAQAPKADNKFNKEQQNAFYEILHLPNLTEEQRNGFIQSLKDDPSVSKEILAEAKKLNDAQAPK

SEQ ID NO: 18 - protein, 305 aa, Peptostreptococcus magnus
AVENKEETPETPETDSEEEVTIKANLIFANGSTQTAEFKGTFEKATSEAYAYADTLKKDNGEYTVDVADKGYTLNIKFAGKEKTPEEPKEEVTIKANLIYADGKTQTAEFKGTFEEATAEAYRYADALKKDNGEYTVDVADKGYTLNIKFAGKEKTPEEPKEEVTIKANLIYADGKTQTAEFKGTFEEATAEAYRYADLLAKENGKYTVDVADKGYTLNIKFAGKEKTPEEPKEEVTIKANLIYADGKTQTAEFKGTFAEATAEAYRYADLLAKENGKYTADLEDGGYTINIRFAGKKVDEKPEE

SEQ ID NO: 19 - protein, 161 aa, Streptococcus sp. G148
AQHDEAVDANSRGSVDASELTPAVTTYKLVINGKTLKGETTTEAVDAATAEKVFKQYANDNGVDGEWTYDDATKTFTVTEKPEVIDASELTPAVTTYKLVINGKTLKGETTTKAVDAETAEKAFKQYANDNGVDGVWTYDDATKTFTVTEMVTEVPLESTA